European Patent Specification EP 4 171 643 B1, published June 4, 2025. Title: THERAPEUTIC COMBINATION OF GALNAC-OLIGONUCLEOTIDE CONJUGATE AND SAPONIN, AND USES THEREOF. Applicant: Sapreme Technologies B.V. The sequence listing filed with the application follows.

SEQUENCE LISTING (18 sequences)

SEQ ID NO: 1 - DNA, 16 bp, Artificial Sequence
  Antisense BNA (HSP27) oligo nucleic acid sequence
ggcacagccagtggcg

SEQ ID NO: 2 - DNA, 20 bp, Artificial Sequence
  APOB BNA oligo
gcctcagtctgcttcgcacc

SEQ ID NO: 3 - DNA, 20 bp, Artificial Sequence
  APOB scrambled BNA oligo
ggcctctctacaccgctcgt

SEQ ID NO: 4 - DNA, 20 bp, Artificial Sequence
  HSP27 primer forward sequence
gcagtccaacgagatcacca

SEQ ID NO: 5 - DNA, 20 bp, Artificial Sequence
  HSP27 primer reverse sequence
taaggctttacttggcggca

SEQ ID NO: 6 - DNA, 20 bp, Artificial Sequence
  ApoB primer forward sequence
agggtccgggaatctgatga

SEQ ID NO: 7 - DNA, 21 bp, Artificial Sequence
  ApoB primer reverse sequence
tgggcacgttgtctttcagag

SEQ ID NO: 8 - DNA, 20 bp, Artificial Sequence
  HBMS primer forward sequence
cacccacacacagcctactt

SEQ ID NO: 9 - DNA, 20 bp, Artificial Sequence
  HBMS primer reverse sequence
gtacccacgcgaatcactct

SEQ ID NO: 10 - DNA, 22 bp, Artificial Sequence
  GUSB primer forward sequence
gaaaatacgtggttggagagct

SEQ ID NO: 11 - DNA, 22 bp, Artificial Sequence
  GUSB primer reverse sequence
ccgagtgaagatccccttttta

SEQ ID NO: 12 - DNA, 13 bp, Artificial Sequence
  ApoB#02
gcattggtattca

SEQ ID NO: 13 - DNA, 24 bp, Artificial Sequence
  ApoB#02 forward primer
gctaacactaagaaccagaagatc

SEQ ID NO: 14 - DNA, 20 bp, Artificial Sequence
  ApoB#02 reverse primer
tgtccgtctaaggatcctgc

SEQ ID NO: 15 - DNA, 18 bp, Artificial Sequence
  Mm PPIA forward primer
gcggcaggtccatctacg

SEQ ID NO: 16 - DNA, 19 bp, Artificial Sequence
  Mm PPIA reverse primer
gccatccagccattcagtc

SEQ ID NO: 17 - DNA, 20 bp, Artificial Sequence
  Mm SDHA forward primer
gaggaagcacaccctctcat

SEQ ID NO: 18 - DNA, 20 bp, Artificial Sequence
  Mm SDHA reverse primer
ggagcggatagcaggaggta